European Patent Specification EP 3 800 196 B1, published July 23, 2025. Title: Peptides for treating rheumatoid arthritis and uses thereof. Applicant: Seoul National University Industry Foundation. The sequence listing filed with the application follows.

SEQUENCE LISTING (5 sequences)

SEQ ID NO: 1 - protein, 12 aa, Artificial Sequence
  peptide #1
AICKEQHLFLPF

SEQ ID NO: 2 - protein, 12 aa, Artificial Sequence
  peptide #2
CKEQHLFLPFSY

SEQ ID NO: 3 - protein, 12 aa, Artificial Sequence
  peptide #3
SYKNKYGMVAQV

SEQ ID NO: 4 - protein, 12 aa, Artificial Sequence
  peptide #4
KNKYGMVAQVTQ

SEQ ID NO: 5 - protein, 12 aa, Artificial Sequence
  peptide #5
TKKMGLAFESTK